European Patent Application EP 4 201 953 A1, published June 28, 2023. Title: IMMUNOCONJUGATES OF AN ANTl-PD-1 ANTIBODY WITH A MUTANT IL-2 OR WITH IL-15. Applicant: F. Hoffmann-La Roche AG. The sequence listing filed with the application follows.

SEQUENCE LISTING (51 sequences)

SEQ ID NO: 1 - protein, 4 aa, synthetic construct
  REGION 1..4: note = Synthetic construct
SSYT

SEQ ID NO: 2 - protein, 8 aa, synthetic construct
  REGION 1..8: note = Synthetic construct
SGGGRDIY

SEQ ID NO: 3 - protein, 5 aa, synthetic construct
  REGION 1..5: note = Synthetic Construct
GRVYF

SEQ ID NO: 4 - protein, 6 aa, synthetic construct
  REGION 1..6: note = Synthetic Construct
TSDNSF

SEQ ID NO: 5 - protein, 7 aa, synthetic construct
  REGION 1..7: note = Synthetic Construct
RSSTLES

SEQ ID NO: 6 - protein, 6 aa, synthetic construct
  REGION 1..6: note = Synthetic Construct
NYDVPW

SEQ ID NO: 7 - skipped

SEQ ID NO: 8 - protein, 7 aa, synthetic construct
  REGION 1..7: note = Synthetic Construct
GFSFSSY

SEQ ID NO: 9 - skipped

SEQ ID NO: 10 - protein, 9 aa, synthetic construct
  REGION 1..9: note = Synthetic Construct
TGRVYFALD

SEQ ID NO: 11 - protein, 11 aa, synthetic construct
  REGION 1..11: note = Synthetic Construct
SESVDTSDNSF

SEQ ID NO: 12 - skipped

SEQ ID NO: 13 - protein, 6 aa, synthetic construct
  REGION 1..6: note = Synthetic Construct
NYDVPW

SEQ ID NO: 14 - protein, 120 aa, synthetic construct
  REGION 1..120: note = Synthetic Construct
EVQLLESGGGLVQPGGSLRLSCAASGFSFSSYTMSWVRQAPGKGLEWVATISGGGRDIYYPDSVKGRFTISRDNSKNTLYLQMNSLRAEDTAVYYCVLLTGRVYFALDSWGQGTLVTVSS

SEQ ID NO: 15 - protein, 111 aa, synthetic construct
  REGION 1..111: note = Synthetic Construct
DIVMTQSPDSLAVSLGERATINCKASESVDTSDNSFIHWYQQKPGQSPKLLIYRSSTLESGVPDRFSGSGSGTDFTLTISSLQAEDVAVYYCQQNYDVPWTFGQGTKVEIK

SEQ ID NO: 16 - protein, 111 aa, synthetic construct
  REGION 1..111: note = Synthetic Construct
DVVMTQSPLSLPVTLGQPASISCRASESVDTSDNSFIHWYQQRPGQSPRLLIYRSSTLESGVPDRFSGSGSGTDFTLKISRVEAEDVGVYYCQQNYDVPWTFGQGTKVEIK

SEQ ID NO: 17 - protein, 111 aa, synthetic construct
  REGION 1..111: note = Synthetic Construct
EIVLTQSPATLSLSPGERATLSCRASESVDTSDNSFIHWYQQKPGQSPRLLIYRSSTLESGIPARFSGSGSGTDFTLTISSLEPEDFAVYYCQQNYDVPWTFGQGTKVEIK

SEQ ID NO: 18 - protein, 111 aa, synthetic construct; identical to SEQ ID NO: 17
  REGION 1..111: note = Synthetic Construct

SEQ ID NO: 19 - protein, 133 aa, Homo sapiens [sequence omitted]

SEQ ID NO: 20 - protein, 133 aa, synthetic construct
  REGION 1..133: note = Synthetic Construct
APASSSTKKTQLQLEHLLLDLQMILNGINNYKNPKLTRMLTAKFAMPKKATELKHLQCLEEELKPLEEVLNGAQSKNFHLRPRDLISNINVIVLELKGSETTFMCEYADETATIVEFLNRWITFAQSIISTLT

SEQ ID NO: 21 - protein, 15 aa, synthetic construct
  REGION 1..15: note = Synthetic Construct
GGGGSGGGGSGGGGS

SEQ ID NO: 22 - protein, 597 aa, synthetic construct
  REGION 1..597: note = Synthetic Construct
EVQLLESGGGLVQPGGSLRLSCAASGFSFSSYTMSWVRQAPGKGLEWVATISGGGRDIYYPDSVKGRFTISRDNSKNTLYLQMNSLRAEDTAVYYCVLLTGRVYFALDSWGQGTLVTVSSASTKGPSVFPLAPSSKSTSGGTAALGCLVKDYFPEPVTVSWNSGALTSGVHTFPAVLQSSGLYSLSSVVTVPSSSLGTQTYICNVNHKPSNTKVDKKVEPKSCDKTHTCPPCPAPEAAGGPSVFLFPPKPKDTLMISRTPEVTCVVVDVSHEDPEVKFNWYVDGVEVHNAKTKPREEQYNSTYRVVSVLTVLHQDWLNGKEYKCKVSNKALGAPIEKTISKAKGQPREPQVYTLPPCRDELTKNQVSLWCLVKGFYPSDIAVEWESNGQPENNYKTTPPVLDSDGSFFLYSKLTVDKSRWQQGNVFSCSVMHEALHNHYTQKSLSLSPGGGGGSGGGGSGGGGSAPASSSTKKTQLQLEHLLLDLQMILNGINNYKNPKLTRMLTAKFAMPKKATELKHLQCLEEELKPLEEVLNGAQSKNFHLRPRDLISNINVIVLELKGSETTFMCEYADETATIVEFLNRWITFAQSIISTLT

SEQ ID NO: 23 - protein, 448 aa, synthetic construct
  REGION 1..448: note = Synthetic Construct
EVQLLESGGGLVQPGGSLRLSCAASGFSFSSYTMSWVRQAPGKGLEWVATISGGGRDIYYPDSVKGRFTISRDNSKNTLYLQMNSLRAEDTAVYYCVLLTGRVYFALDSWGQGTLVTVSSASTKGPSVFPLAPSSKSTSGGTAALGCLVKDYFPEPVTVSWNSGALTSGVHTFPAVLQSSGLYSLSSVVTVPSSSLGTQTYICNVNHKPSNTKVDKKVEPKSCDKTHTCPPCPAPEAAGGPSVFLFPPKPKDTLMISRTPEVTCVVVDVSHEDPEVKFNWYVDGVEVHNAKTKPREEQYNSTYRVVSVLTVLHQDWLNGKEYKCKVSNKALGAPIEKTISKAKGQPREPQVCTLPPSRDELTKNQVSLSCAVKGFYPSDIAVEWESNGQPENNYKTTPPVLDSDGSFFLVSKLTVDKSRWQQGNVFSCSVMHEALHNHYTQKSLSLSP

SEQ ID NO: 24 - protein, 448 aa, synthetic construct
  REGION 1..448: note = Synthetic Construct
EVQLLESGGGLVQPGGSLRLSCAASGFSFSSYTMSWVRQAPGKGLEWVATISGGGRDIYYPDSVKGRFTISRDNSKNTLYLQMNSLRAEDTAVYYCVLLTGRVYFALDSWGQGTLVTVSSASTKGPSVFPLAPSSKSTSGGTAALGCLVKDYFPEPVTVSWNSGALTSGVHTFPAVLQSSGLYSLSSVVTVPSSSLGTQTYICNVNHKPSNTKVDKKVEPKSCDKTHTCPPCPAPEAAGGPSVFLFPPKPKDTLMISRTPEVTCVVVDVSHEDPEVKFNWYVDGVEVHNAKTKPREEQYNSTYRVVSVLTVLHQDWLNGKEYKCKVSNKALGAPIEKTISKAKGQPREPQVCTLPPSRDELTKNQVSLSCAVKGFYPSDIAVEWESNGQPENNYKTTPPVLDSDGSFFLVSKLTVDKSRWQQGNVFSCSVMHEALHNRFTQKSLSLSP

SEQ ID NO: 25 - protein, 218 aa, synthetic construct
  REGION 1..218: note = Synthetic Construct
DIVMTQSPDSLAVSLGERATINCKASESVDTSDNSFIHWYQQKPGQSPKLLIYRSSTLESGVPDRFSGSGSGTDFTLTISSLQAEDVAVYYCQQNYDVPWTFGQGTKVEIKRTVAAPSVFIFPPSDEQLKSGTASVVCLLNNFYPREAKVQWKVDNALQSGNSQESVTEQDSKDSTYSLSSTLTLSKADYEKHKVYACEVTHQGLSSPVTKSFNRGEC

SEQ ID NO: 26 - protein, 20 aa, Homo sapiens
MYRMQLLSCIALSLALVTNS

SEQ ID NO: 27 - protein, 268 aa, Homo sapiens
PGWFLDSPDRPWNPPTFSPALLVVTEGDNATFTCSFSNTSESFVLNWYRMSPSNQTDKLAAFPEDRSQPGQDCRFRVTQLPNGRDFHMSVVRARRNDSGTYLCGAISLAPKAQIKESLRAELRVTERRAEVPTAHPSPSPRPAGQFQTLVVGVVGGLLGSLVLLVWVLAVICSRAARGTIGARRTGQPLKEDPSAVPVFSVDYGELDFQWREKTPEPPVPCVPEQTEYATIVFPSGMGTSSPARRGSADGPRSAQPLRPEDGHCSWPL

SEQ ID NO: 28 - protein, 288 aa, Homo sapiens
MQIPQAPWPVVWAVLQLGWRPGWFLDSPDRPWNPPTFSPALLVVTEGDNATFTCSFSNTSESFVLNWYRMSPSNQTDKLAAFPEDRSQPGQDCRFRVTQLPNGRDFHMSVVRARRNDSGTYLCGAISLAPKAQIKESLRAELRVTERRAEVPTAHPSPSPRPAGQFQTLVVGVVGGLLGSLVLLVWVLAVICSRAARGTIGARRTGQPLKEDPSAVPVFSVDYGELDFQWREKTPEPPVPCVPEQTEYATIVFPSGMGTSSPARRGSADGPRSAQPLRPEDGHCSWPL

SEQ ID NO: 29 - protein, 133 aa, synthetic construct
  REGION 1..133: note = Synthetic Construct
APTSSSTKKTQLQLEHLLLDLQMILNGINNYKNPKLTRMLTFKFYMPKKATELKHLQCLEEELKPLEEVLNLAQSKNFHLRPRDLISNINVIVLELKGSETTFMCEYADETATIVEFLNRWITFAQSIISTLT

SEQ ID NO: 30 - protein, 225 aa, Homo sapiens
DKTHTCPPCPAPELLGGPSVFLFPPKPKDTLMISRTPEVTCVVVDVSHEDPEVKFNWYVDGVEVHNAKTKPREEQYNSTYRVVSVLTVLHQDWLNGKEYKCKVSNKALPAPIEKTISKAKGQPREPQVYTLPPSRDELTKNQVSLTCLVKGFYPSDIAVEWESNGQPENNYKTTPPVLDSDGSFFLYSKLTVDKSRWQQGNVFSCSVMHEALHNHYTQKSLSLSP

SEQ ID NO: 31 - protein, 107 aa, Homo sapiens [sequence omitted]

SEQ ID NO: 32 - protein, 105 aa, Homo sapiens
QPKAAPSVTLFPPSSEELQANKATLVCLISDFYPGAVTVAWKADSSPVKAGVETTTPSKQSNNKYAASSYLSLTPEQWKSHRSYSCQVTHEGSTVEKTVAPTECS

SEQ ID NO: 33 - protein, 328 aa, Homo sapiens
ASTKGPSVFPLAPSSKSTSGGTAALGCLVKDYFPEPVTVSWNSGALTSGVHTFPAVLQSSGLYSLSSVVTVPSSSLGTQTYICNVNHKPSNTKVDKKVEPKSCDKTHTCPPCPAPELLGGPSVFLFPPKPKDTLMISRTPEVTCVVVDVSHEDPEVKFNWYVDGVEVHNAKTKPREEQYNSTYRVVSVLTVLHQDWLNGKEYKCKVSNKALPAPIEKTISKAKGQPREPQVYTLPPSRDELTKNQVSLTCLVKGFYPSDIAVEWESNGQPENNYKTTPPVLDSDGSFFLYSKLTVDKSRWQQGNVFSCSVMHEALHNHYTQKSLSLSP

SEQ ID NO: 34 - protein, 607 aa, synthetic construct
  REGION 1..607: note = Synthetic Construct
EVQLQESGPGLVKPSQSLSLTCSVTGYSITSSYRWNWIRKFPGNRLEWMGYINSAGISNYNPSLKRRISITRDTSKNQFFLQVNSVTTEDAATYYCARSDNMGTTPFTYWGQGTLVTVSSAKTTPPSVYPLAPGSAAQTNSMVTLGCLVKGYFPEPVTVTWNSGSLSSGVHTFPAVLQSDLYTLSSSVTVPSSTWPSQTVTCNVAHPASSTKVDKKIVPRDCGCKPCICTVPEVSSVFIFPPKPKDVLTITLTPKVTCVVVAISKDDPEVQFSWFVDDVEVHTAQTKPREEQINSTFRSVSELPIMHQDWLNGKEFKCRVNSAAFGAPIEKTISKTKGRPKAPQVYTIPPPKEQMAKDKVSLTCMITNFFPEDITVEWQWNGQPAENYDNTQPIMDTDGSYFVYSDLNVQKSNWEAGNTFTCSVLHEGLHNHHTEKSLSHSPGGGGGSGGGGSGGGGSAPASSSTSSSTAEAQQQQQQQQQQQQHLEQLLMDLQELLSRMENYRNLKLPRMLTAKFALPKQATELKDLQCLEDELGPLRHVLDGTQSKSFQLEDAENFISNIRVTVVKLKGSDNTFECQFDDESATVVDFLRRWIAFAQSIISTSPQ

SEQ ID NO: 35 - protein, 442 aa, synthetic construct
  REGION 1..442: note = Synthetic Construct
EVQLQESGPGLVKPSQSLSLTCSVTGYSITSSYRWNWIRKFPGNRLEWMGYINSAGISNYNPSLKRRISITRDTSKNQFFLQVNSVTTEDAATYYCARSDNMGTTPFTYWGQGTLVTVSSAKTTPPSVYPLAPGSAAQTNSMVTLGCLVKGYFPEPVTVTWNSGSLSSGVHTFPAVLQSDLYTLSSSVTVPSSTWPSQTVTCNVAHPASSTKVDKKIVPRDCGCKPCICTVPEVSSVFIFPPKPKDVLTITLTPKVTCVVVAISKDDPEVQFSWFVDDVEVHTAQTKPREEQINSTFRSVSELPIMHQDWLNGKEFKCRVNSAAFGAPIEKTISKTKGRPKAPQVYTIPPPKKQMAKDKVSLTCMITNFFPEDITVEWQWNGQPAENYKNTQPIMKTDGSYFVYSKLNVQKSNWEAGNTFTCSVLHEGLHNHHTEKSLSHSP

SEQ ID NO: 36 - protein, 218 aa, synthetic construct
  REGION 1..218: note = Synthetic Construct
DIVMTQGTLPNPVPSGESVSITCRSSKSLLYSDGKTYLNWYLQRPGQSPQLLIYWMSTRASGVSDRFSGSGSGTDFTLKISGVEAEDVGIYYCQQGLEFPTFGGGTKLELKRTDAAPTVSIFPPSSEQLTSGGASVVCFLNNFYPKDINVKWKIDGSERQNGVLNSWTDQDSKDSTYSMSSTLTLTKDEYERHNSYTCEATHKTSTSPIVKSFNRNEC

SEQ ID NO: 37 - protein, 595 aa, synthetic construct
  REGION 1..595: note = Synthetic Construct
EVQLVESGGGLVQPGGSLRLSCAASGFTFSDSWIHWVRQAPGKGLEWVAWISPYGGSTYYADSVKGRFTISADTSKNTAYLQMNSLRAEDTAVYYCARRHWPGGFDYWGQGTLVTVSAASTKGPSVFPLAPSSKSTSGGTAALGCLVKDYFPEPVTVSWNSGALTSGVHTFPAVLQSSGLYSLSSVVTVPSSSLGTQTYICNVNHKPSNTKVDKKVEPKSCDKTHTCPPCPAPEAAGGPSVFLFPPKPKDTLMISRTPEVTCVVVDVSHEDPEVKFNWYVDGVEVHNAKTKPREEQYNSTYRVVSVLTVLHQDWLNGKEYKCKVSNKALGAPIEKTISKAKGQPREPQVYTLPPCRDELTKNQVSLWCLVKGFYPSDIAVEWESNGQPENNYKTTPPVLDSDGSFFLYSKLTVDKSRWQQGNVFSCSVMHEALHNHYTQKSLSLSPGGGGGSGGGGSGGGGSAPASSSTKKTQLQLEHLLLDLQMILNGINNYKNPKLTRMLTAKFAMPKKATELKHLQCLEEELKPLEEVLNGAQSKNFHLRPRDLISNINVIVLELKGSETTFMCEYADETATIVEFLNRWITFAQSIISTLT

SEQ ID NO: 38 - protein, 446 aa, synthetic construct
  REGION 1..446: note = Synthetic Construct
EVQLVESGGGLVQPGGSLRLSCAASGFTFSDSWIHWVRQAPGKGLEWVAWISPYGGSTYYADSVKGRFTISADTSKNTAYLQMNSLRAEDTAVYYCARRHWPGGFDYWGQGTLVTVSAASTKGPSVFPLAPSSKSTSGGTAALGCLVKDYFPEPVTVSWNSGALTSGVHTFPAVLQSSGLYSLSSVVTVPSSSLGTQTYICNVNHKPSNTKVDKKVEPKSCDKTHTCPPCPAPEAAGGPSVFLFPPKPKDTLMISRTPEVTCVVVDVSHEDPEVKFNWYVDGVEVHNAKTKPREEQYNSTYRVVSVLTVLHQDWLNGKEYKCKVSNKALGAPIEKTISKAKGQPREPQVCTLPPSRDELTKNQVSLSCAVKGFYPSDIAVEWESNGQPENNYKTTPPVLDSDGSFFLVSKLTVDKSRWQQGNVFSCSVMHEALHNHYTQKSLSLSP

SEQ ID NO: 39 - protein, 214 aa, synthetic construct
  REGION 1..214: note = Synthetic Construct
DIQMTQSPSSLSASVGDRVTITCRASQDVSTAVAWYQQKPGKAPKLLIYSASFLYSGVPSRFSGSGSGTDFTLTISSLQPEDFATYYCQQYLYHPATFGQGTKVEIKRTVAAPSVFIFPPSDEQLKSGTASVVCLLNNFYPREAKVQWKVDNALQSGNSQESVTEQDSKDSTYSLSSTLTLSKADYEKHKVYACEVTHQGLSSPVTKSFNRGEC

SEQ ID NO: 40 - protein, 605 aa, synthetic construct
  REGION 1..605: note = Synthetic Construct
EVQLVESGGGLVQPGGSLRLSCAASGFTFSDSWIHWVRQAPGKGLEWVAWISPYGGSTYYADSVKGRFTISADTSKNTAYLQMNSLRAEDTAVYYCARRHWPGGFDYWGQGTLVTVSAAKTTPPSVYPLAPGSAAQTNSMVTLGCLVKGYFPEPVTVTWNSGSLSSGVHTFPAVLQSDLYTLSSSVTVPSSTWPSETVTCNVAHPASSTKVDKKIVPRDCGCKPCICTVPEVSSVFIFPPKPKDVLTITLTPKVTCVVVAISKDDPEVQFSWFVDDVEVHTAQTQPREEQFNSTFRSVSELPIMHQDWLNGKEFKCRVNSAAFGAPIEKTISKTKGRPKAPQVYTIPPPKEQMAKDKVSLTCMITDFFPEDITVEWQWNGQPAENYDNTQPIMDTDGSYFVYSDLNVQKSNWEAGNTFTCSVLHEGLHNHHTEKSLSHSPGGGGGSGGGGSGGGGSAPASSSTSSSTAEAQQQQQQQQQQQQHLEQLLMDLQELLSRMENYRNLKLPRMLTAKFALPKQATELKDLQCLEDELGPLRHVLDGTQSKSFQLEDAENFISNIRVTVVKLKGSDNTFECQFDDESATVVDFLRRWIAFAQSIISTSPQ

SEQ ID NO: 41 - protein, 440 aa, synthetic construct
  REGION 1..440: note = Synthetic Construct
EVQLVESGGGLVQPGGSLRLSCAASGFTFSDSWIHWVRQAPGKGLEWVAWISPYGGSTYYADSVKGRFTISADTSKNTAYLQMNSLRAEDTAVYYCARRHWPGGFDYWGQGTLVTVSAAKTTPPSVYPLAPGSAAQTNSMVTLGCLVKGYFPEPVTVTWNSGSLSSGVHTFPAVLQSDLYTLSSSVTVPSSTWPSETVTCNVAHPASSTKVDKKIVPRDCGCKPCICTVPEVSSVFIFPPKPKDVLTITLTPKVTCVVVAISKDDPEVQFSWFVDDVEVHTAQTQPREEQFNSTFRSVSELPIMHQDWLNGKEFKCRVNSAAFGAPIEKTISKTKGRPKAPQVYTIPPPKKQMAKDKVSLTCMITDFFPEDITVEWQWNGQPAENYKNTQPIMKTDGSYFVYSKLNVQKSNWEAGNTFTCSVLHEGLHNHHTEKSLSHSP

SEQ ID NO: 42 - protein, 214 aa, synthetic construct
  REGION 1..214: note = Synthetic Construct
DIQMTQSPSSLSASVGDRVTITCRASQDVSTAVAWYQQKPGKAPKLLIYSASFLYSGVPSRFSGSGSGTDFTLTISSLQPEDFATYYCQQYLYHPATFGQGTKVEIKRADAAPTVSIFPPSSEQLTSGGASVVCFLNNFYPKDINVKWKIDGSERQNGVLNSWTDQDSKDSTYSMSSTLTLTKDEYERHNSYTCEATHKTSTSPIVKSFNRNEC

SEQ ID NO: 43 - protein, 150 aa, Homo sapiens [sequence omitted]

SEQ ID NO: 44 - protein, 608 aa, synthetic construct
  REGION 1..608: note = Synthetic Construct
QVQLVQSGAEVKKPGASVKVSCKASGYTFTEFGMNWVRQAPGQGLEWMGWINTKTGEATYVEEFKGRVTFTTDTSTSTAYMELRSLRSDDTAVYYCARWDFAYYVEAMDYWGQGTTVTVSSAKTTPPSVYPLAPGSAAQTNSMVTLGCLVKGYFPEPVTVTWNSGSLSSGVHTFPAVLQSDLYTLSSSVTVPSSTWPSQTVTCNVAHPASSTKVDKKIVPRDCGCKPCICTVPEVSSVFIFPPKPKDVLTITLTPKVTCVVVAISKDDPEVQFSWFVDDVEVHTAQTKPREEQINSTFRSVSELPIMHQDWLNGKEFKCRVNSAAFGAPIEKTISKTKGRPKAPQVYTIPPPKEQMAKDKVSLTCMITNFFPEDITVEWQWNGQPAENYDNTQPIMDTDGSYFVYSDLNVQKSNWEAGNTFTCSVLHEGLHNHHTEKSLSHSPGGGGGSGGGGSGGGGSAPASSSTSSSTAEAQQQQQQQQQQQQHLEQLLMDLQELLSRMENYRNLKLPRMLTAKFALPKQATELKDLQCLEDELGPLRHVLDGTQSKSFQLEDAENFISNIRVTVVKLKGSDNTFECQFDDESATVVDFLRRWIAFAQSIISTSPQ

SEQ ID NO: 45 - protein, 445 aa, synthetic construct
  REGION 1..445: note = Synthetic Construct
QVQLVQSGAEVKKPGASVKVSCKASGYTFTEFGMNWVRQAPGQGLEWMGWINTKTGEATYVEEFKGRVTFTTDTSTSTAYMELRSLRSDDTAVYYCARWDFAYYVEAMDYWGQGTTVTVSSAKTTPPSVYPLAPGSAAQTNSMVTLGCLVKGYFPEPVTVTWNSGSLSSGVHTFPAVLQSDLYTLSSSVTVPSSTWPSQTVTCNVAHPASSTKVDKKIVPRDCGCKPCICTVPEVSSVFIFPPKPKDVLTITLTPKVTCVVVAISKDDPEVQFSWFVDDVEVHTAQTKPREEQINSTFRSVSELPIMHQDWLNGKEFKCRVNSAAFGAPIEKTISKTKGRPKAPQVYTIPPPKKQMAKDKVSLTCMITNFFPEDITVEWQWNGQPAENYKNTQPIMKTDGSYFVYSKLNVQKSNWEAGNTFTCSVLHEGLHNHHTEKSLSHSPGK

SEQ ID NO: 46 - protein, 215 aa, synthetic construct
  REGION 1..215: note = Synthetic Construct
DIQMTQSPSSLSASVGDRVTITCKASAAVGTYVAWYQQKPGKAPKLLIYSASYRKRGVPSRFSGSGSGTDFTLTISSLQPEDFATYYCHQYYTYPLFTFGQGTKLEIKRADAAPTVSIFPPSSEQLTSGGASVVCFLNNFYPKDINVKWKIDGSERQNGVLNSWTDQDSKDSTYSMSSTLTLTKDEYERHNSYTCEATHKTSTSPIVKSFNRNEC

SEQ ID NO: 47 - protein, 604 aa, synthetic construct
  REGION 1..604: note = Synthetic Construct
EVQLLESGGGLVQPGGSLRLSCAASGFTFSSYAMSWVRQAPGKGLEWVSAIIGSGASTYYADSVKGRFTISRDNSKNTLYLQMNSLRAEDTAVYYCAKGWFGGFNYWGQGTLVTVSSAKTTPPSVYPLAPGSAAQTNSMVTLGCLVKGYFPEPVTVTWNSGSLSSGVHTFPAVLQSDLYTLSSSVTVPSSTWPSQTVTCNVAHPASSTKVDKKIVPRDCGCKPCICTVPEVSSVFIFPPKPKDVLTITLTPKVTCVVVAISKDDPEVQFSWFVDDVEVHTAQTKPREEQINSTFRSVSELPIMHQDWLNGKEFKCRVNSAAFGAPIEKTISKTKGRPKAPQVYTIPPPKEQMAKDKVSLTCMITNFFPEDITVEWQWNGQPAENYDNTQPIMDTDGSYFVYSDLNVQKSNWEAGNTFTCSVLHEGLHNHHTEKSLSHSPGGGGGSGGGGSGGGGSAPASSSTSSSTAEAQQQQQQQQQQQQHLEQLLMDLQELLSRMENYRNLKLPRMLTAKFALPKQATELKDLQCLEDELGPLRHVLDGTQSKSFQLEDAENFISNIRVTVVKLKGSDNTFECQFDDESATVVDFLRRWIAFAQSIISTSPQ

SEQ ID NO: 48 - protein, 441 aa, synthetic construct
  REGION 1..441: note = Synthetic Construct
EVQLLESGGGLVQPGGSLRLSCAASGFTFSSYAMSWVRQAPGKGLEWVSAIIGSGASTYYADSVKGRFTISRDNSKNTLYLQMNSLRAEDTAVYYCAKGWFGGFNYWGQGTLVTVSSAKTTPPSVYPLAPGSAAQTNSMVTLGCLVKGYFPEPVTVTWNSGSLSSGVHTFPAVLQSDLYTLSSSVTVPSSTWPSQTVTCNVAHPASSTKVDKKIVPRDCGCKPCICTVPEVSSVFIFPPKPKDVLTITLTPKVTCVVVAISKDDPEVQFSWFVDDVEVHTAQTKPREEQINSTFRSVSELPIMHQDWLNGKEFKCRVNSAAFGAPIEKTISKTKGRPKAPQVYTIPPPKKQMAKDKVSLTCMITNFFPEDITVEWQWNGQPAENYKNTQPIMKTDGSYFVYSKLNVQKSNWEAGNTFTCSVLHEGLHNHHTEKSLSHSPGK

SEQ ID NO: 49 - protein, 215 aa, synthetic construct
  REGION 1..215: note = Synthetic Construct
EIVLTQSPGTLSLSPGERATLSCRASQSVTSSYLAWYQQKPGQAPRLLINVGSRRATGIPDRFSGSGSGTDFTLTISRLEPEDFAVYYCQQGIMLPPTFGQGTKVEIKRADAAPTVSIFPPSSEQLTSGGASVVCFLNNFYPKDINVKWKIDGSERQNGVLNSWTDQDSKDSTYSMSSTLTLTKDEYERHNSYTCEATHKTSTSPIVKSFNRNEC

SEQ ID NO: 50 - protein, 450 aa, synthetic construct
  REGION 1..450: note = Synthetic Construct
EVQLQESGPGLVKPSQSLSLTCSVTGYSITSSYRWNWIRKFPGNRLEWMGYINSAGISNYNPSLKRRISITRDTSKNQFFLQVNSVTTEDAATYYCARSDNMGTTPFTYWGQGTLVTVSSASTTAPSVYPLAPVCGDTTGSSVTLGCLVKGYFPEPVTLTWNSGSLSSGVHTFPAVLQSDLYTLSSSVTVTSSTWPSQSITCNVAHPASSTKVDKKIEPRGPTIKPCPPCKCPAPNAAGGPSVFIFPPKIKDVLMISLSPIVTCVVVDVSEDDPDVQISWFVNNVEVHTAQTQTHREDYNSTLRVVSALPIQHQDWMSGKEFKCKVNNKDLGAPIERTISKPKGSVRAPQVYVLPPPEEEMTKKQVTLTCMVTDFMPEDIYVEWTNNGKTELNYKNTEPVLDSDGSYFMYSKLRVEKKNWVERNSYSCSVVHEGLHNHHTTKSFSRTPGK

SEQ ID NO: 51 - protein, 218 aa, synthetic construct; identical to SEQ ID NO: 36
  REGION 1..218: note = Synthetic Construct